European Patent Application EP 4 219 486 A1, published August 2, 2023. Title: Novel Bridged Bicycloalkyl-Substituted Aminothiazoles and Their Methods of Use. Applicant: Temple University of The Commonwealth System Of Higher Education. The sequence listing filed with the application follows.

SEQUENCE LISTING (16 sequences)

SEQ ID NO: 1 - RNA, 21 nt, synthetic construct
  misc_feature 1..21: note = chemically synthesized
  source 1..21: mol_type = other RNA
ggattgccctgagctaatttt

SEQ ID NO: 2 - skipped

SEQ ID NO: 3 - protein, 23 aa, synthetic construct
  REGION 1..23: note = chemically synthesized
KIPDPDSDDVSEVDARHIIENAK

SEQ ID NO: 4 - protein, 20 aa, synthetic construct
  REGION 1..20: note = chemically synthesized
YKDSSSGRQLSEVFIQLPSR

SEQ ID NO: 5 - DNA, 23 bp, synthetic construct
  misc_feature 1..23: note = chemically synthesized
  source 1..23: mol_type = other DNA
gaattcagtgccactaagcagac

SEQ ID NO: 6 - DNA, 23 bp, synthetic construct
  misc_feature 1..23: note = chemically synthesized
  source 1..23: mol_type = other DNA
tcggtatatccaagacatgatcc

SEQ ID NO: 7 - DNA, 24 bp, synthetic construct
  misc_feature 1..24: note = chemically synthesized
  source 1..24: mol_type = other DNA
atatccctcaccacgatcctaata

SEQ ID NO: 8 - DNA, 24 bp, synthetic construct
  misc_feature 1..24: note = chemically synthesized
  source 1..24: mol_type = other DNA
ccctctgtagtgcaaagactgata

SEQ ID NO: 9 - DNA, 23 bp, synthetic construct
  misc_feature 1..23: note = chemically synthesized
  source 1..23: mol_type = other DNA
tcttggagtcctcactcaaactc

SEQ ID NO: 10 - DNA, 23 bp, synthetic construct
  misc_feature 1..23: note = chemically synthesized
  source 1..23: mol_type = other DNA
actgctgcaactacccttaaaca

SEQ ID NO: 11 - DNA, 23 bp, synthetic construct
  misc_feature 1..23: note = chemically synthesized
  source 1..23: mol_type = other DNA
caggaaactaactttcagccaga

SEQ ID NO: 12 - DNA, 23 bp, synthetic construct
  misc_feature 1..23: note = chemically synthesized
  source 1..23: mol_type = other DNA
taaagagggcatggagtaattga

SEQ ID NO: 13 - DNA, 20 bp, synthetic construct
  misc_feature 1..20: note = chemically synthesized
  source 1..20: mol_type = other DNA
tctcacaatcctggaggctg

SEQ ID NO: 14 - DNA, 20 bp, synthetic construct
  misc_feature 1..20: note = chemically synthesized
  source 1..20: mol_type = other DNA
gaccaagaagcaagccctca

SEQ ID NO: 15 - DNA, 19 bp, synthetic construct
  misc_feature 1..19: note = chemically synthesized
  source 1..19: mol_type = other DNA
cagacagacactggcaaca

SEQ ID NO: 16 - DNA, 19 bp, synthetic construct
  misc_feature 1..19: note = chemically synthesized
  source 1..19: mol_type = other DNA
acatctcccccttctcctt